European Patent Specification EP 4 077 357 B1, published September 6, 2023. Title: BINDING PROTEINS FOR THE ENZYME ACID ALPHA-GLUCOSIDASE AND USES THEREOF. Applicant: Navigo Proteins GmbH. The sequence listing filed with the application follows.

SEQUENCE LISTING (23 sequences)

SEQ ID NO: 1 - protein, 58 aa, Artificial Sequence
  GAA binding protein (monomer)
IAAKFDMKQAWADHFILELPNLTEEQRNAFRQSLSDDPSVSDLVLLQAQKLNQMQAPK

SEQ ID NO: 2 - protein, 58 aa, Artificial Sequence
  GAA binding protein
IAAKFDMKQAWADHFILELPNLTEEQRNAFRQSLSDDPSVSDLVLAQAQKLNQSQAPK

SEQ ID NO: 3 - protein, 59 aa, Artificial Sequence
  GAA binding protein (with C-terminal Cys)
IAAKFDMKQAWADHFILELPNLTEEQRNAFRQSLSDDPSVSDLVLLQAQKLNQMQAPKC

SEQ ID NO: 4 - protein, 59 aa, Artificial Sequence
  GAA binding protein (C-terminal Cys)
IAAKFDMKQAWADHFILELPNLTEEQRNAFRQSLSDDPSVSDLVLAQAQKLNQSQAPKC

SEQ ID NO: 5 - protein, 65 aa, Artificial Sequence
  GAA binding protein (N-cap and C-terminal Cys)
VDAKFDIAAKFDMKQAWADHFILELPNLTEEQRNAFRQSLSDDPSVSDLVLLQAQKLNQMQAPKC

SEQ ID NO: 6 - protein, 65 aa, Artificial Sequence
  GAA binding protein (N-cap and C-terminal Cys)
VDAKFDIAAKFDMKQAWADHFILELPNLTEEQRNAFRQSLSDDPSVSDLVLAQAQKLNQSQAPKC

SEQ ID NO: 7 - protein, 116 aa, Artificial Sequence
  GAA binding protein (dimer)
IAAKFDMKQAWADHFILELPNLTEEQRNAFRQSLSDDPSVSDLVLLQAQKLNQMQAPKIAAKFDMKQAWADHFILELPNLTEEQRNAFRQSLSDDPSVSDLVLLQAQKLNQMQAPK

SEQ ID NO: 8 - protein, 117 aa, Artificial Sequence
  GAA binding protein (dimer with C-terminal Cys)
IAAKFDMKQAWADHFILELPNLTEEQRNAFRQSLSDDPSVSDLVLLQAQKLNQMQAPKIAAKFDMKQAWADHFILELPNLTEEQRNAFRQSLSDDPSVSDLVLLQAQKLNQMQAPKC

SEQ ID NO: 9 - protein, 174 aa, Artificial Sequence
  Fusion protein GAA binding protein
IAAKFDEAQQAADYEILHLPNLTEEQRNAFRQSLRDDPSVSLEVLGEAQKLNDSQAPKIAAKFDMKQAWADHFILELPNLTEEQRNAFRQSLSDDPSVSDLVLLQAQKLNQMQAPKIAAKFDEAQQAADYEILHLPNLTEEQRNAFRQSLRDDPSVSLEVLGEAQKLNDSQAPK

SEQ ID NO: 10 - protein, 58 aa, Artificial Sequence
  non Fc binding protein; scaffold protein
IAAKFDEAQSAADSEILHLPNLTEEQRNAFRQSLSDDPSVSLEVLGEAQKLNDSQAPK

SEQ ID NO: 11 - protein, 58 aa, Artificial Sequence
  non-Fc binding protein
IAAKFDEAQQAADYEILHLPNLTEEQRNAFRQSLRDDPSVSLEVLGEAQKLNDSQAPK

SEQ ID NO: 12 - protein, 10 aa, Artificial Sequence
  Streptag
SAWSHPQFEK

SEQ ID NO: 13 - protein, 8 aa, Artificial Sequence
  flag-tag
DYKDDDDK

SEQ ID NO: 14 - protein, 174 aa, Artificial Sequence
  204870 cor1-PAdelFc2-PAdelFc2
IAAKFDMKQAWADHFILELPNLTEEQRNAFRQSLSDDPSVSDLVLLQAQKLNQMQAPKIAAKFDEAQQAADYEILHLPNLTEEQRNAFRQSLRDDPSVSLEVLGEAQKLNDSQAPKIAAKFDEAQQAADYEILHLPNLTEEQRNAFRQSLRDDPSVSLEVLGEAQKLNDSQAPK

SEQ ID NO: 15 - protein, 232 aa, Artificial Sequence
  core1 dimer - PAdelFc2 dimer
IAAKFDMKQAWADHFILELPNLTEEQRNAFRQSLSDDPSVSDLVLLQAQKLNQMQAPKIAAKFDMKQAWADHFILELPNLTEEQRNAFRQSLSDDPSVSDLVLLQAQKLNQMQAPKIAAKFDEAQQAADYEILHLPNLTEEQRNAFRQSLRDDPSVSLEVLGEAQKLNDSQAPKIAAKFDEAQQAADYEILHLPNLTEEQRNAFRQSLRDDPSVSLEVLGEAQKLNDSQAPK

SEQ ID NO: 16 - protein, 56 aa, Artificial Sequence
  GAA binding protein
AKFDMKQAWADHFILELPNLTEEQRNAFRQSLSDDPSVSDLVLLQAQKLNQMQAPK

SEQ ID NO: 17 - protein, 56 aa, Artificial Sequence
  GAA binding protein
AKFDMKQAWADHFILELPNLTEEQRNAFRQSLSDDPSVSDLVLAQAQKLNQSQAPK

SEQ ID NO: 18 - protein, 46 aa, Artificial Sequence
  GAA binding protein
  Xaa (38)..(38): Xaa may be selected from any amino acid
  Xaa (46)..(46): Xaa may be selected from any amino acid
QAWADHFILELPNLTEEQRNAFRQSLSDDPSVSDLVLXQAQKLNQX

SEQ ID NO: 19 - protein, 171 aa, Artificial Sequence
  fusion protein comprising GAA binding protein
AKFDMKQAWADHFILELPNLTEEQRNAFRQSLSDDPSVSDLVLLQAQKLNQMQAPKAQHDKDQQAADKEILHLPNLTEEQRNKFRQSLRDDPSVSAEILAEAKKLNDAQAPKIAAQHDKDQQAADKEILHLPNLTEEQRNKFRQSLRDDPSVSAEILAEAKKLNDAQAPKC

SEQ ID NO: 20 - protein, 171 aa, Artificial Sequence
  fusion protein comprising GAA binding protein
AKFDMKQAWADHFILELPNLTEEQRNAFRQSLSDDPSVSDLVLAQAQKLNQSQAPKAQHDKDQQAADKEILHLPNLTEEQRNKFRQSLRDDPSVSAEILAEAKKLNDAQAPKIAAQHDKDQQAADKEILHLPNLTEEQRNKFRQSLRDDPSVSAEILAEAKKLNDAQAPKC

SEQ ID NO: 21 - protein, 58 aa, Artificial Sequence
  non Ig binding protein
IAAQHDKIQQAADKEILHLPNLTEEQRNKFRQSLRDDPSVSAEILAEAKKLNDAQAPK

SEQ ID NO: 22 - protein, 46 aa, Artificial Sequence
  GAA binding protein
QAWADHFILELPNLTEEQRNAFRQSLSDDPSVSDLVLLQAQKLNQM

SEQ ID NO: 23 - protein, 46 aa, Artificial Sequence
  GAA binding protein
QAWADHFILELPNLTEEQRNAFRQSLSDDPSVSDLVLAQAQKLNQS